European Patent Specification EP 3 541 959 B1, published June 24, 2026. Title: COMPOSITIONS AND METHODS FOR DETECTING OR QUANTIFYING HEPATITIS B VIRUS. Applicant: GEN-PROBE INCORPORATED GAO, Kui LINNEN, Jeffrey M. The sequence listing filed with the application follows.

SEQUENCE LISTING (125 sequences)

SEQ ID NO: 1 - DNA, 3221 bp, Hepatitis B virus
  ref <308>: AB116092
  ref <309>: 2006-10-05
  ref <313>: (1)..(3221)
ttccacagctttccaccaagctctgcaagatcccagagtcaggggcctgtattttcctgctggtggctccagttcaggaacactcaaccctgttccaactattgcctctcacatctcgtcaatctcctcgaggattggggaccctgcaccgaacatggagaacatcacatcaggattcctaggacccctgctcgtgttacaggcggggtttttcttgttgacaagaatcctcacaataccgcagagtctagactcgtggtggacttctctcaattttctagggggagcacccgtgtgtcttggccaaaattcgcagtccccaacctccaatcactcaccaacctcctgtcctccaatttgtcctggttatcgctggatgtgtctgcggcgttttatcatattcctcttcatcctgctgctatgcctcatcttcttattggttcttctggattatcaaggtatgttgcccgtttgtcctctaattccaggatcaacaacaaccagcacgggaccctgcaaaacctgcacgactcctgctcaagggaactctatgtttccctcatgttgctgtacaaaacctacggatggaaattgcacctgtattcccatcccatcatcttggggtttcgcaaaattcctatgggagtgggcctcagtccgtttctcttgtctcagtttactagtgccatttgttcagtggttcgtagggctttcccccactgtttggcttttagctatatggatgatgtggtactgggggccaagtctgtacaacatcttgagtccctttacaccgctgttaccaattttcttttgtctttgggtatacatttaaaccctaacaaaacaaagagatggggttattccctgaatttcatgggttatgtaattggaagttggggtacattgccacaggatcatattgtacaaaaaatcaaacactgttttagaaaacttcctgtaaatcgacctattgattggaaagtatgtcagagaattgtgggtcttttgggctttgcagctccatttacacaatgtggttaccctgcattaatgcctttgtatgcatgtatacaggcgaaacaggcttttactttctcgccaacttacaaggcctttctaagtaaacagtatatgaacctttaccccgttgcccggcaacggcctggtctgtgccaagtgtttgctgacgcaacccccactggctggggcttggccatcggccatcagcgcatgcgtggaacctttgtggctcctctgccgatccatactgcggaactcctagccgcttgttttgctcgcagcaggtctggagcaaaactcatcggaactgataattctgtcgtcctttctcggaagtatacatcctttccatggctgctaggttgtactgccaactggattcttcgcgggacgtcctttgtctacgtcccgtcggcgctgaatcccgcggacgacccttcgcgaggccgcttggggctgtatcgtccccttctccgtctgccgtaccgtccgaccacggggcgcacctctctttacgcggtctccccgtctgtgccttctcatctgccggtccgtgtgcacttcgcttcacctctgcacgttgcatggagaccaccgtgaacgcccatcaggtcctgcccaaggtcttatataagaggactcttggactctcagcaatgtcaacgaccgaccttgaggcctacttcaaagactgtgtgtttaaagactgggaggagttgggggaggagattaggttaatgatctttgtattaggaggctgtaggcataaattggtctgcgcaccatcatcatgcaactttttcacctctgcctaatcatctcttgtacatgtcccacttttcaagcctccaagctgtgccttggatggctttggggcatggacattgacccttataaagaatttggagctactgtggagttactttcatttttgccttctgacttctttccttccgtccgggatctactagatacagtcgcagctctatttcgggatgccttagagtctcctgagcattgctcagctcaccacacagcactaaggcaagtcattctctgctggggggaattaatgactctagctacctgggtgggtactaatttgcaagatccagcatccagggatctagtagtcagttatgttaatgataacatgggcctaaagatcaggcaattattatggtttcatacttcttgcattacttttggaagagaaactgtccttgagtatttggtctctttcggagtgtggattcgcactcctccagcctatagaccaccaaatgcccctatcttatcaacacttccggaaactactgttgttagacgacgagaccgaggcaggtcccctagaagaagaactccctcgcctcgcagacgaagatctcaatcgccgcgtcgcagaagatctcaatctcgggaacctcaatgttagtattccttggactcataaggtgggaaattttactggactttattcttctactgtccctatctttaatcctgaatggcaaacaccgtcttttcctaaaattcatttacatgaagacattgctaataggtgtcagcaatttgtaggccctctcactgtaaatgaaaaaagaagactgaaattaattatgcctgctaggttttatcctaacagcacaaaatatttgcctttagacaaagggattaaaacttattatcctgatcaggtagttaatcattactttcaaacccgacattatttacatactctttggaaggctgggattctatataagagggaaactacacgtagcgcctcatattgcgggtcaccatattcttgggaacaagagctacatcatgggaggttggtcatcaaaacctcgcaaaggcatggggacgaacctttctgttcccaacccgctgggattctttcccgatcatcagttggaccctgcattcggagccaatgcaaacaatccagattgggacctcaaccccatcaaggaccactggccacaagccaaccaggtaggagtgggagcatttggaccagggctcactcccccacacggaggtgttttggggtggagccctcaggctcaaggcatattggccaccgtgccaacagtgcctcctcctgcctccaccaatcggcagtcgggaaggcagcctactcccatttctccacctctaagagacagtcatcctcaggccatgcagtggaa

SEQ ID NO: 2 - DNA, 23 bp, Artificial Sequence
  Synthetic Oligomer
ggcacctagtccagaagaaccaa

SEQ ID NO: 3 - DNA, 21 bp, Artificial Sequence
  Synthetic Oligomer
ggcacctagtccagaagaacc

SEQ ID NO: 4 - DNA, 10 bp, Artificial Sequence
  Synthetic Oligomer
cagaagaacc

SEQ ID NO: 5 - DNA, 10 bp, Artificial Sequence
  Synthetic Oligomer
tagtccagaa

SEQ ID NO: 6 - DNA, 10 bp, Artificial Sequence
  Synthetic Oligomer
gcacctagtc

SEQ ID NO: 7 - DNA, 10 bp, Artificial Sequence
  Synthetic Oligomer
gaagaaccaa

SEQ ID NO: 8 - DNA, 18 bp, Artificial Sequence
  Synthetic Oligomer
taatacgactcactatag

SEQ ID NO: 9 - DNA, 23 bp, Artificial Sequence
  Synthetic Oligomer
taatacgactcactatagggaga

SEQ ID NO: 10 - DNA, 31 bp, Artificial Sequence
  Synthetic Oligomer
taatacgactcactatagggagaccacaacg

SEQ ID NO: 11 - DNA, 22 bp, Artificial Sequence
  Synthetic Oligomer
aatttaatacgactcactatag

SEQ ID NO: 12 - DNA, 27 bp, Artificial Sequence
  Synthetic Oligomer
aatttaatacgactcactatagggaga

SEQ ID NO: 13 - DNA, 35 bp, Artificial Sequence
  Synthetic Oligomer
aatttaatacgactcactatagggagaccacaacg

SEQ ID NO: 14 - DNA, 49 bp, Artificial Sequence
  Synthetic Oligomer
aatttaatacgactcactatagggagagatgtgtctgcggcgttttatc

SEQ ID NO: 15 - DNA, 54 bp, Artificial Sequence
  Synthetic Oligomer
aatttaatacgactcactatagggagagatgtgtctgcggcgttttatcatctt

SEQ ID NO: 16 - DNA, 57 bp, Artificial Sequence
  Synthetic Oligomer
aatttaatacgactcactatagggagagatgtgtctgcggcgttttatcatcttcct

SEQ ID NO: 17 - DNA, 35 bp, Artificial Sequence
  Synthetic Oligomer
ggagagatgtgtctgcggcgttttatcatcttcct

SEQ ID NO: 18 - DNA, 27 bp, Artificial Sequence
  Synthetic Oligomer
ggagagatgtgtctgcggcgttttatc

SEQ ID NO: 19 - DNA, 32 bp, Artificial Sequence
  Synthetic Oligomer
ggagagatgtgtctgcggcgttttatcatctt

SEQ ID NO: 20 - DNA, 30 bp, Artificial Sequence
  Synthetic Oligomer
gatgtgtctgcggcgttttatcatcttcct

SEQ ID NO: 21 - DNA, 22 bp, Artificial Sequence
  Synthetic Oligomer
gatgtgtctgcggcgttttatc

SEQ ID NO: 22 - DNA, 27 bp, Artificial Sequence
  Synthetic Oligomer
gatgtgtctgcggcgttttatcatctt

SEQ ID NO: 23 - DNA, 10 bp, Artificial Sequence
  Synthetic Oligomer
gcgttttatc

SEQ ID NO: 24 - DNA, 10 bp, Artificial Sequence
  Synthetic Oligomer
ctgcggcgtt

SEQ ID NO: 25 - DNA, 10 bp, Artificial Sequence
  Synthetic Oligomer
tgtgtctgcg

SEQ ID NO: 26 - DNA, 10 bp, Artificial Sequence
  Synthetic Oligomer
ttatcatctt

SEQ ID NO: 27 - DNA, 10 bp, Artificial Sequence
  Synthetic Oligomer
tcatcttcct

SEQ ID NO: 28 - DNA, 10 bp, Artificial Sequence
  Synthetic Oligomer
ggagagatgt

SEQ ID NO: 29 - RNA, 38 nt, Artificial Sequence
  Synthetic oligomer
  misc_feature (33)..(34): Non-nucleotide c9 linker inserted between base positions 33-34
cccacaagaagaugaggcauagcagcaggaugaguggg

SEQ ID NO: 30 - DNA, 56 bp, Artificial Sequence
  Synthetic Oligomer
aatttaatacgactcactatagggagaccacaacggtgggcctcagtccgtttctc

SEQ ID NO: 31 - DNA, 62 bp, Artificial Sequence
  Synthetic Oligomer
  misc_feature (57)..(57): n = Inosine
aatttaatacgactcactatagggagaccacaacggtgggcctcagtccgtttctcntggct

SEQ ID NO: 32 - DNA, 34 bp, Artificial Sequence
  Synthetic Oligomer
ggagaccacaacggtgggcctcagtccgtttctc

SEQ ID NO: 33 - DNA, 40 bp, Artificial Sequence
  Synthetic Oligomer
  misc_feature (35)..(35): n = Inosine
ggagaccacaacggtgggcctcagtccgtttctcntggct

SEQ ID NO: 34 - DNA, 29 bp, Artificial Sequence
  Synthetic Oligomer
ccacaacggtgggcctcagtccgtttctc

SEQ ID NO: 35 - DNA, 35 bp, Artificial Sequence
  Synthetic Oligomer
  misc_feature (30)..(30): n = Inosine
ccacaacggtgggcctcagtccgtttctcntggct

SEQ ID NO: 36 - DNA, 10 bp, Artificial Sequence
  Synthetic Oligomer
tccgtttctc

SEQ ID NO: 37 - DNA, 10 bp, Artificial Sequence
  Synthetic Oligomer
ctcagtccgt

SEQ ID NO: 38 - DNA, 10 bp, Artificial Sequence
  Synthetic Oligomer
tgggcctcag

SEQ ID NO: 39 - DNA, 10 bp, Artificial Sequence
  Synthetic Oligomer
  misc_feature (5)..(5): n = Inosine
tctcntggct

SEQ ID NO: 40 - RNA, 26 nt, Artificial Sequence
  Synthetic oligomer
  misc_feature (21)..(22): Non-nucleotide c9 linker inserted between base positions 21-22
ugcgcuaguaaacugagccaggcgca

SEQ ID NO: 41 - DNA, 20 bp, Artificial Sequence
  Synthetic Oligomer
cctgcgaaccactgaacaaa

SEQ ID NO: 42 - DNA, 11 bp, Artificial Sequence
  Synthetic Oligomer
cactgaacaaa

SEQ ID NO: 43 - DNA, 10 bp, Artificial Sequence
  Synthetic Oligomer
gaaccactga

SEQ ID NO: 44 - DNA, 10 bp, Artificial Sequence
  Synthetic Oligomer
cctgcgaacc

SEQ ID NO: 45 - DNA, 58 bp, Artificial Sequence
  Synthetic Oligomer
  misc_feature (26)..(58): Immobilized probe-binding region: Tail
gggctttcccccactgtttggcttttttaaaaaaaaaaaaaaaaaaaaaaaaaaaaaa

SEQ ID NO: 46 - DNA, 58 bp, Artificial Sequence
  Synthetic Oligomer
  misc_feature (26)..(58): Immobilized probe-binding region: Tail
agttatatggatgatgtggtattggtttaaaaaaaaaaaaaaaaaaaaaaaaaaaaaa

SEQ ID NO: 47 - DNA, 59 bp, Artificial Sequence
  Synthetic Oligomer
  misc_feature (27)..(59): Immobilized probe-binding region: Tail
ggtctgtgccaagtgtttgctgacgctttaaaaaaaaaaaaaaaaaaaaaaaaaaaaaa

SEQ ID NO: 48 - DNA, 58 bp, Artificial Sequence
  Synthetic Oligomer
  misc_feature (29)..(58): Immobilized probe-binding region: Tail
ttgttttgctcgcagccggtctggagcgaaaaaaaaaaaaaaaaaaaaaaaaaaaaaa

SEQ ID NO: 49 - DNA, 22 bp, Artificial Sequence
  Synthetic Oligomer
gggctttcccccactgtttggc

SEQ ID NO: 50 - DNA, 10 bp, Artificial Sequence
  Synthetic Oligomer
actgtttggc

SEQ ID NO: 51 - DNA, 10 bp, Artificial Sequence
  Synthetic Oligomer
cccccactgt

SEQ ID NO: 52 - DNA, 10 bp, Artificial Sequence
  Synthetic Oligomer
gggctttccc

SEQ ID NO: 53 - DNA, 25 bp, Artificial Sequence
  Synthetic Oligomer
agttatatggatgatgtggtattgg

SEQ ID NO: 54 - DNA, 10 bp, Artificial Sequence
  Synthetic Oligomer
gtggtattgg

SEQ ID NO: 55 - DNA, 10 bp, Artificial Sequence
  Synthetic Oligomer
atgatgtggt

SEQ ID NO: 56 - DNA, 10 bp, Artificial Sequence
  Synthetic Oligomer
tatggatgat

SEQ ID NO: 57 - DNA, 26 bp, Artificial Sequence
  Synthetic Oligomer
ggtctgtgccaagtgtttgctgacgc

SEQ ID NO: 58 - DNA, 10 bp, Artificial Sequence
  Synthetic Oligomer
ttgctgacgc

SEQ ID NO: 59 - DNA, 10 bp, Artificial Sequence
  Synthetic Oligomer
agtgtttgct

SEQ ID NO: 60 - DNA, 10 bp, Artificial Sequence
  Synthetic Oligomer
tgccaagtgt

SEQ ID NO: 61 - DNA, 28 bp, Artificial Sequence
  Synthetic Oligomer
ttgttttgctcgcagccggtctggagcg

SEQ ID NO: 62 - DNA, 10 bp, Artificial Sequence
  Synthetic Oligomer
gtctggagcg

SEQ ID NO: 63 - DNA, 10 bp, Artificial Sequence
  Synthetic Oligomer
agccggtctg

SEQ ID NO: 64 - DNA, 10 bp, Artificial Sequence
  Synthetic Oligomer
ctcgcagccg

SEQ ID NO: 65 - DNA, 33 bp, Artificial Sequence
  Synthetic Oligomer
tttaaaaaaaaaaaaaaaaaaaaaaaaaaaaaa

SEQ ID NO: 66 - DNA, 30 bp, Artificial Sequence
  Synthetic Oligomer
aaaaaaaaaaaaaaaaaaaaaaaaaaaaaa

SEQ ID NO: 67 - DNA, 57 bp, Artificial Sequence
  Synthetic Oligomer
aatttaatacgactcactatagggagaagactcgtggtggacttctctcaattttct

SEQ ID NO: 68 - DNA, 35 bp, Artificial Sequence
  Synthetic Oligomer
ggagaagactcgtggtggacttctctcaattttct

SEQ ID NO: 69 - DNA, 30 bp, Artificial Sequence
  Synthetic Oligomer
agactcgtggtggacttctctcaattttct

SEQ ID NO: 70 - DNA, 10 bp, Artificial Sequence
  Synthetic Oligomer
tcaattttct

SEQ ID NO: 71 - DNA, 10 bp, Artificial Sequence
  Synthetic Oligomer
ttctctcaat

SEQ ID NO: 72 - DNA, 10 bp, Artificial Sequence
  Synthetic Oligomer
tggacttctc

SEQ ID NO: 73 - DNA, 20 bp, Artificial Sequence
  Synthetic Oligomer
tatcaaggtatgttgcccgt

SEQ ID NO: 74 - DNA, 10 bp, Artificial Sequence
  Synthetic Oligomer
tgttgcccgt

SEQ ID NO: 75 - DNA, 10 bp, Artificial Sequence
  Synthetic Oligomer
aggtatgttg

SEQ ID NO: 76 - DNA, 10 bp, Artificial Sequence
  Synthetic Oligomer
tatcaaggta

SEQ ID NO: 77 - DNA, 19 bp, Artificial Sequence
  Synthetic Oligomer
gattatataggacgacaag

SEQ ID NO: 78 - DNA, 49 bp, Artificial Sequence
  Synthetic Oligomer
aatttaatacgactcactatagggagagatgattgacttgtgattccgc

SEQ ID NO: 79 - RNA, 23 nt, Artificial Sequence
  Synthetic oligomer
  misc_feature (5)..(6): Non-nucleotide c9 linker inserted between base positions 5-6
gcauggugcgaauugggacaugc

SEQ ID NO: 80 - DNA, 57 bp, Artificial Sequence
  Synthetic Oligomer
  misc_feature (25)..(57): Immobilized probe-binding region: Tail
cguucacuauuggucucugcauuctttaaaaaaaaaaaaaaaaaaaaaaaaaaaaaa

SEQ ID NO: 81 - RNA, 24 nt, Artificial Sequence
  Synthetic oligomer
cguucacuauuggucucugcauuc

SEQ ID NO: 82 - RNA, 28 nt, Artificial Sequence
  Synthetic oligomer
aagaagaugaggcauagcagcaggauga

SEQ ID NO: 83 - RNA, 10 nt, Artificial Sequence
  Synthetic oligomer
gcuaguaaac

SEQ ID NO: 84 - RNA, 16 nt, Artificial Sequence
  Synthetic oligomer
uaguaaacugagccag

SEQ ID NO: 85 - RNA, 20 nt, Artificial Sequence
  Synthetic oligomer
  misc_feature (18)..(19): Non-nucleotide c9 linker inserted between base positions 18-19
gcuaguaaacugagccaggc

SEQ ID NO: 86 - DNA, 22 bp, Artificial Sequence
  Synthetic Oligomer
gatgattgacttgtgattccgc

SEQ ID NO: 87 - DNA, 59 bp, Artificial Sequence; identical to SEQ ID NO: 47
  Synthetic Oligomer
  misc_feature (27)..(59): Immobilized probe-binding region: Tail

SEQ ID NO: 88 - DNA, 60 bp, Artificial Sequence
  Synthetic Oligomer
  misc_feature (31)..(60): Immobilized probe-binding region: Tail
tcctctgccgatccatactgcggaactcctaaaaaaaaaaaaaaaaaaaaaaaaaaaaaa

SEQ ID NO: 89 - DNA, 58 bp, Artificial Sequence; identical to SEQ ID NO: 48
  Synthetic Oligomer
  misc_feature (29)..(58): Immobilized probe-binding region: Tail

SEQ ID NO: 90 - DNA, 56 bp, Artificial Sequence
  Synthetic Oligomer
  misc_feature (24)..(56): Immobilized probe-binding region: Tail
gggctttcccccactgtttggcttttaaaaaaaaaaaaaaaaaaaaaaaaaaaaaa

SEQ ID NO: 91 - DNA, 58 bp, Artificial Sequence; identical to SEQ ID NO: 46
  Synthetic Oligomer
  misc_feature (26)..(58): Immobilized probe-binding region: Tail

SEQ ID NO: 92 - DNA, 58 bp, Artificial Sequence
  Synthetic Oligomer
  misc_feature (26)..(58): Immobilized probe-binding region: Tail
ccgctgttaccaattttcttttgtctttaaaaaaaaaaaaaaaaaaaaaaaaaaaaaa

SEQ ID NO: 93 - DNA, 59 bp, Artificial Sequence
  Synthetic Oligomer
  misc_feature (27)..(59): Immobilized probe-binding region: Tail
ggucugugccaaguguuugcugacgctttaaaaaaaaaaaaaaaaaaaaaaaaaaaaaa

SEQ ID NO: 94 - DNA, 58 bp, Artificial Sequence
  Synthetic Oligomer
  misc_feature (26)..(58): Immobilized probe-binding region: Tail
gucugugccaaguguuugcugacgctttaaaaaaaaaaaaaaaaaaaaaaaaaaaaaa

SEQ ID NO: 95 - DNA, 58 bp, Artificial Sequence
  Synthetic Oligomer
  misc_feature (26)..(58): Immobilized probe-binding region: Tail
aguuauauggaugaugugguauuggtttaaaaaaaaaaaaaaaaaaaaaaaaaaaaaa

SEQ ID NO: 96 - DNA, 26 bp, Artificial Sequence
  Synthetic Oligomer
ggtctgtgccaagtgtttgctgacgc

SEQ ID NO: 97 - DNA, 29 bp, Artificial Sequence
  Synthetic Oligomer
tcctctgccgatccatactgcggaactcc

SEQ ID NO: 98 - DNA, 28 bp, Artificial Sequence
  Synthetic Oligomer
ttgttttgctcgcagccggtctggagcg

SEQ ID NO: 99 - DNA, 26 bp, Artificial Sequence
  Synthetic Oligomer
gggctttcccccactgtttggctttt

SEQ ID NO: 100 - DNA, 25 bp, Artificial Sequence
  Synthetic Oligomer
agttatatggatgatgtggtattgg

SEQ ID NO: 101 - DNA, 25 bp, Artificial Sequence
  Synthetic Oligomer
ccgctgttaccaattttcttttgtc

SEQ ID NO: 102 - DNA, 26 bp, Artificial Sequence
  Synthetic Oligomer
ggucugugccaaguguuugcugacgc

SEQ ID NO: 103 - DNA, 25 bp, Artificial Sequence
  Synthetic Oligomer
gucugugccaaguguuugcugacgc

SEQ ID NO: 104 - DNA, 25 bp, Artificial Sequence
  Synthetic Oligomer
aguuauauggaugaugugguauugg

SEQ ID NO: 105 - DNA, 960 bp, Hepatitis B virus
  ref <308>: AY707087
  ref <309>: 2007-10-23
  ref <313>: (1)..(900)
aattccactgccttccaccaagctctgcaggatcccaaagtcaggggtctgtattttcctgctggtggctccagttcaggaacagtaaaccctgctccgaatattgcctctcacatctcgtcaatctccgcgaggactggggaccctgtgacgaatatggagaacatcacatcaggattcctaggacccctgctcgtgttacaggcggggtttttcttgttgacaagaatcctcacaataccgcagagtctagactcgtggtggacttctctcaattttctagggggatcacccgtgtgtcttggccaaaattcgcagtccccaacctccaatcactcaccaacctcctgtcctccaatttgtcctggttatcgctggatgtgtctgcggcgttttatcatattcctcttcatcctgctgctatgcctcatcttcttgttggttcttctggattatcaaggtatgttgcccgtttgtcctctaattccaggaacaacaacaaccagtacgggaccatgcaaaacctgcacgactcctgctcaaggcaactctatgtttccctcatgttgctgtacaaaaccttcggatggaaattgcacctgtattcccatcccatcgtcttgggctttcgcaaaatacctatgggagtgggcctcagtccgtttctcttggctcagtttactagtgccatttgttcagtggttcgtagggctttcccccactgtttggctttcagctatatggatgatgtggtattgggggccaagtctgtacagcatcgtgagtccctttataccgctgttaccaattttcttttgtctctgggtatacatttaaaccctaacaaaacaaaaagatggggttattccctaaacttcatgggttacataattggaagttggggaacgttgccacaggatcatattgtacaaaagatcaaacactgttttagaaaacttc

SEQ ID NO: 106 - DNA, 900 bp, Hepatitis B virus
  ref <308>: AB194951
  ref <309>: 2007-11-17
  ref <313>: (1)..(900)
ttccacaaatttccaccaagctctgcaagatcccagagtcaggggcctgtatcttcctgctggtggctccagttcaggaacagtcaaccctgctccgaatattgcctctcacatctcgtcaatctcctcgaggattggggaccctgcgccgaacatggagaacatcacatcaggattcctaggacccctgctcgtgttacaggcggggtttttctcgttgacaaaaatcctcacaataccgcagagtctagactcgtggtggacttctctcaattttctagggggagcacccgtgtgtcttggccaaaattcgcagtccccaacctccaatcactcaccaacctcctgtcctccaatttgtcctggttatcgctggatgtgtctgcggcgttttatcatattcctcttcatcctgctgctatgcctcatcttcttattggttcttctggattgtcaaggtatgttgcccgtttgtcctctaattccaggatccacaaccaccagtacgggaccctgcagaacctgcacgactcctgctcaaggcaactctatgtttccctcatgttgctgtacaaaacctacggacggaaattgcacctgtattcccatcccatcatcctgggctttcgcaaaatacctatgggggtgggcctcagtccgtttctcctggctcagtttactagtgccatttgttcagtggttcgtagggctttcccccattgtttggctttcagctatatggatgatgtggtattgggggccaagtctgtacaacatcttgagtccctttataccgctgttaccaattttcttttggctttgggcatacatttaaaccctaacaaaacaaaaagatggggttattcccttaacttcatgggatacataattggaagttgg

SEQ ID NO: 107 - DNA, 900 bp, Hepatitis B virus
  ref <308>: AB014366
  ref <309>: 2006-11-02
  ref <313>: (1)..(900)
ttccaccactttccaccaaactcttcaagatcccagagtcagggctctgtaccttcctgctggtggctccagttcaggaatagtaagccctgctcagaatactgtctctgccatatcgtcaatcttatcgacgactggggaccctgtgccgaacatggagaacatcgcatcaggactcctaggacccctgctcgtgttacaggcggggtttttctcgttgacaaaaatcctcacaataccacagagtctagactcgtggtggacttctctcagttttctagggggaacacccgtgtgtcttggccaaaattcgcagtcccaaatctccagtcactcaccaacctgttgtcctccaatttgtcctggttatcgctggatgtatctgcggcgttttatcatctgcctctgcatcctgctgctatgcctcatcttcttgttggttcttctggactatcaaggtatgttgcccgtttgtcctctaattccaggatcatcaaccaccagcacgggaccatgcaagacctgcacaactcctgctcaaggaacctctatgtttccctcatgttgctgtacaaaacctacggacggaaactgcacctgtattcccatcccatcatcttgggctttcgcaaaattcctatgggagtgggcctcagtccgtttctcttggctcagtttactagtgccatttgttcagtggttcgtagggctttcccccactgtctggctttcagttatatggatgatgtggtattgggggccaagtctgtacaacatcttgagtccctttatgccgctgttaccaattttcttttgtctttgggtatacatttaaaccctcacaaaacaaaaagatggggatattcccttaatttcatgggatatgtaattgggagttgg

SEQ ID NO: 108 - DNA, 900 bp, Hepatitis B virus
  ref <308>: AY596111
  ref <309>: 2004-08-24
  ref <313>: (1)..(900)
ctccaccactttccaccaaactcttcaagatcccagagtcagggccctgtactttcctgctggtggctccagttcaggaacagtgagccctgctcagaatactgtctctgccatatcgtcaatcttatcgaagactggggaccctgtaccgaacatggagaacatcgcatcaggactcctaggacccctgctcgtgttacaggcggggtttttctcgttgacaaaaatcctcacaataccacagagtctagactcgtggtggacttctctcagttttctaggggaaacacccgtgtgtcttggccaaaattcgcagtcccaaatctccagtcactcaccaacctgttgtcctccaatttgtcctggttatcgctggatgtgtctgcggcgttttatcatcttcctctgcatcctgctgctatgcctcatcttcttgttggttcttctggactatcaaggtatgttgcccgtttgtcctctaattccaggatcatcaacaaccagcaccggaccatgcaaaacctgcacaacttctgctcaaggaacctctatgtttccctcatgttgctgtacaaaacctacggacggaaactgcacctgtattcccatcccatcatcttgggctttcgcaaaatacctatgggagtgggcctcagtccgtttctcttggctcagtttactagtgccatttgttcagtggttcgtagggctttcccccactgtctggctttcagttatatggatgatgtggttttgggggccaagactgtacagcatcttgagtccctttatgccgctgttaccaattttcttttgtctttgggcatacatttaaaccctcacaaaacaaaaagatggggatattcccttaacttcatgggatatgtaattgggagttgg

SEQ ID NO: 109 - DNA, 900 bp, Hepatitis B virus
  ref <308>: M54923
  ref <309>: 2000-06-13
  ref <313>: (1)..(900)
ctccaccacgttccaccaaactcttcaagatcccagagtcagggctctgtactttcctgctggtggctccagttcaggaacagtaaaccctgttcagaacactgtctcttccatatcgtcaatcttatcgaagactggggaccctgtgccgaacatggagaacatcgcatcaggactcctaggacccctgctcgtgttacaggcggggtttttcttgttgacaaaaatcctcacaataccacagagtctagactcgtggtggacttctctcaattttctagggggaacacccgtgtgtcttggccaaaattcgcagtcccaaatctccagtcactcaccaacttgttgtcctccgatttgtcctggttatcgctggatgtgtctgcggcgttttatcatcttcctctgcatcctgctgctatgcctcatcttcttgttggttcttctggactatcaaggtatgttgcccgtttgtcctctaattccaggatcatcaaccaccagcaccggaccatgcaaaacctgcacgactcctgctcaaggaacctctatgtttccctcatgttgctgtacaaaacctacggacggaaactgcacctgtattcccatcccatcatcttgggctttcgcaaaatacctatgggagtgggcctcagtccgtttctcttggctcagtttactagtgccatttgttcagtggttcgtagggctttcccccactgtctggctttcagttatatggatgatgtggttttgggggccaagtctgtacaacatcttgagtccctttatgccgctgttaccaattttcttttgtctttgggtatacatttaaaccctcagaaaacaaaaagatggggctactccctcaacttcatggggtatgtaattggaagttgg

SEQ ID NO: 110 - DNA, 900 bp, Hepatitis B virus
  ref <308>: AB073835
  ref <309>: 2002-06-04
  ref <313>: (1)..(900)
ctccaccactttccatcaaactcttcaagatcccagagtcagggctctgtactttcctgctggtggctccagttcaggaatagtaaaccctgctcagaatactgcctctgccatatcatcaaccttctcgaagactggggaccctgtaccgaacatggagaacatcgcatcaggactcctaggacccctgctcgtgttacaggcggggtttttctcgttgacaaaaatcctcacaataccacagagtctagactcgtggtggacttctctcaattttctagggggaacacccgtgtgtcttggccaaaattcgcagtcccaaatctccagtcactcaccaacttgttgtcctccaacttgtcctggttatcgctggatgtatctgcggcgttttatcatattcctctgcatcctgctgctatgcctcatcttcttgttggttcttctggactatcaaggtatgttgcccgtttgtcctctaattccaggatcatcaaccaccagcaccggaccctgcagaacctgcacgactcctgctcaaggaacctctatgtttccctcatgttgctgtacaaaacctacggacggaaactgcacctgtattcccatcccatcatcttgggctttcgcaaaattcctatgggagtgggcctcagtccgtttctcttggctcagtttactagtgccgtttgttcagtggttcgtagggctttcccccactgtctggctttcagttatatggatgatgtggtattgggggccaaatctgtacaacatcttgagtccctttatgccgctgttaccaattttcttttgtctttgggtatacatttaaaccctcacaaaacaaaaagatggggatattcccttaatttcatgggatatgtaattggtagttgg

SEQ ID NO: 111 - DNA, 900 bp, Hepatitis B virus
  ref <308>: AY123424
  ref <309>: 2002-08-16
  ref <313>: (1)..(900)
aactccacaacattccaccaagctctgctagaccccagagtgaggggcctatactttcctgctggtggctccagttccggaacagtaaaccctgttccgactactgcctcacccatatcgtcaatcttctcgaggactggggaccctgcaccgaacatggagagcacaacatcaggattcctaggacccctgctcgtgttacaggcggggtttttcttgttgacaagaatcctcacaataccacagagtctagactcgtggtggacttctctcaattttctagggggagcacccacgtgtcttggccaaaattcgcagtccccaacctccaatcactcaccaacctcttgtcctccaatttgtcctggttatcgttggatgtgtctgcggcgttttatcatattcctcttcatcctgctgctatgcctcatcttcttgttggttcttctggactaccaaggtatgttgcccgtttgtcctctacttccaagaacatcaactaccagcacgggaccatgcaagacctgcacgattcctgctcaaggaacctctatgtttccctcttgttgctgtacaaaaccttcggacggaaactgcacttgtattcccatcccatcatcttgggctttcgcaagattcctatgggagtgggcctcagtccgtttctcctggctcagtttactagtgccatttgttcagtggttcgtagggctttcccccactgtttggctttcagttatatggatgatgtggtattgggggccaagtctgtacaacatcttgagtccctttttacctctattaccaattttcttttgtctttgggtatacatttgaaccccaataaaaccaaacgttggggctattcccttaatttcatgggatatgtaattggatgtt

SEQ ID NO: 112 - DNA, 900 bp, Hepatitis B virus
  ref <308>: AF223955
  ref <309>: 2001-09-07
  ref <313>: (1)..(900)
ctccagcacattccaccaagctctgctagatcccagagtgaggggcctatactttcctgctggtggctccagttccggaacagtaaaccctgttccgactactgcctctcccatatcgtcaatcttctcgaggactggggaccctgcaccgaatatggagagcaccacatcaggattcctaggacccctgctcgtgttacaggcggggtttttcttgttgacaagaatcctcacaataccacagagtctagactcgtggtggacttctctcaattttctagggggagcacccacgtgtcctggccaaaatttgcagtccccaacctccaatcactcaccaacctcttgtcctccaatttgtcctggttatcgctggatgtgtctgcggcgttttatcatcttcctcttcatcctgctgctatgcctcatcttcttgttggttcttctggactaccaaggtatgttgcccgtttgtcctctacttccaggaacatcaactaccagcacgggaccatgcaggacctgcacgattcctgctcaaggaacctctatgtttccctcttgttgctgtacaaaaccttcggacggaaattgcacttgtattcccatcccatcatcttgggctttcgcaagattcctatgggagtgggcctcagtccgtttctcctggctcagtttactagtgccatttgttcagtggttcgtagggctttcccccactgtttggctttcagttatatggatgatgtggtattgggggccaagtctgtacaacatcttgaatccctttttaccgctattaccaattttcttttgtctttgggtatacatttaaaccctaataaaaccaaacgttggggctactcccttaactttatgggatatgtcattggaagttgg

SEQ ID NO: 113 - DNA, 900 bp, Hepatitis B virus
  ref <308>: X75665
  ref <309>: 2006-11-14
  ref <313>: (1)..(900)
ctccacaacattccaacaagctctgcaggatcccagagtcagggtcctttattttcctgctggtggctccagttccggaacagtaaaccctgttccgactactgcctctctcatttcgtcaatcttctcgaggattggggaccctgtaacgaacatggagaacacaacatcaggattcctaggacccctgctcgtgttacaggcggggtttttcttgttgacaaaaatcctcacaataccacagagtctagactcgtggtggacttctctcaattttctagggggagcacccgtgtgtcctggccaaaattcgcagtccccaacctccaatcactcaccaacctcttgtcctccaatttgtcctggctatcgctggatgtgtctgcggcgttttatcatcttcctcttcatcctgctgctatgcctcatcttcttgttggttcttctggactaccaaggtatgttgcccgtttgtcctctacttccaggaacatcaactaccagcacgggaccatgcaagacctgcacgattcctgctcaaggaacctctatgtttccctcatgttgctgtacaaaaccttcggacggaaactgcacttgtattcccatcccatcatcctgggctttcgtaagattcctatgggagtgggcctcagtccgtttctcctggctcagtttactagcgccatttgttcagtggttcgtagggctttcccccactgtttggctttcagttatatggatgatgtggtattgggggccaagtctgtacaacatcttgagtccctttatacctctattaccaattttcttttgtctttgggtatacatttaaaccctaataaaaccaaaagatggggctattcccttaacttcatgggctatgtaattggaagttgg

SEQ ID NO: 114 - DNA, 900 bp, Hepatitis B virus
  ref <308>: AB104712
  ref <309>: 2003-06-26
  ref <313>: (1)..(900)
aactccactaccttccaccaaactctgcaagatcccagagtgagaggcctgtatttccctgctggtggctccagttcaggaacagtaaaccctgttccgactactgtctctcacatatcgtcaatcttctcgaggattggggaccctgcgctgaacatggagaacatcacatcaggattcctaggacccctgctcgtgttacaggcggggtttttcttgttgacaagaatcctcacaataccgcagagtctagactcgtggtggacttctctcaattttctagggggaactaccgtgtgtcttggccaaaattcgcagtccccaacctccaatcactcaccaacctcctgtcctccaacttgtcctggttatcgctggatgtgtctgcggcgttttatcatcttcctcttcatcctgctgctatgcctcatcttcttgttggttcttctggactatcaaggtatgttgcccgtttgtcctctaattccaggatcttcaactaccagcacgggaccatgcagaacctgcacgactcctgctcaaggaacctctatgtatccctcctgctgctgtaccaaaccttcggacggaaattgcacctgtattcccatcccatcatcctgggctttcggaaaattcctatgggagtgggcctcagcccgtttctcctggctcagtttactagtgccatttgttcagtggttcgtagggctttcccccactgtttggctttcagttatatggatgatgtggtattgggggccaagtctgtacagcatcttgagtccctttttaccgctgttaccaattttcttttgtctttgggtatacatttaaaccctaacaaaacaaaaagatggggttactctttacatttcatgggttatgtcattggatgtt

SEQ ID NO: 115 - DNA, 900 bp, Hepatitis B virus; identical to SEQ ID NO: 114
  ref <308>: AB205126
  ref <309>: 2008-11-14
  ref <313>: (1)..(900)

SEQ ID NO: 116 - DNA, 900 bp, Hepatitis B virus
  ref <308>: AY233291
  ref <309>: 2004-04-23
  ref <313>: (1)..(900)
ttccacaaccttccaccaaactctgcaagatcccagagtgagaggcctgtatttccctgctggtggctccagttcaggaacagtaaaccctgttccgactactgcctctcccttatcgtcaatcttctcgaggattggggaccctgcgccgaacatggagaacatcacatcaggattcctaggacccctgctcgtgttacaggcggggtttttcttgttgacaagaatcctcacaataccgcagagtctagactcgtggtggacttctctcaattttctagggggaactaccgtgtgtcttggccaaaattcgcagtccccaacctccaatcactcaccaacctcctgtcctccaacttgtcctggttatcgctggatgtgtctgcggcgttttatcatcttcctcttcatcctgctgctatgcctcatcttcttgttggttcttctggactatcaaggtatgttgcccgtgtgtcctctaattccaggatcctcaaccaccagcacgggaccatgccgaacctgcacgactcctgctcaaggaacctctatgtatccctcctgttgctgtaccaaaccttcggacggaaattgcacctgtattcccatcccatcatcctggcctttcggaaaattcctatgggagtgggcctcagcccgtttctcctggctcagtttactagtgccatttgttcagtggttcgtagggctttcccccactgtttggctttcagttatatggatgatgtggtattgggggccaagtctgtacagcatcttgagtccctttttaccgctgttaccaattttcttttgtctttgggtatacatttaaaccctaacaaaacaaagagatggggttactctctaaattttatggggtatgtcattggatgttat

SEQ ID NO: 117 - DNA, 900 bp, Hepatitis B virus
  ref <308>: AB048702
  ref <309>: 2001-03-23
  ref <313>: (1)..(900)
ctccacaaccttccaccaaactctgcaagatcccagagtgagaggcctgtatctccctgctggtggctccagttcaggaacagtaaaccctgttccgactactgcctctcccatatcgtcaatcttctcgaggattggggaccttgcgctgaacatggagaacatcacatcaggattcctaggacccctgctcgtgttacaggcggggtttttcttgttgacaagaatcctcacaataccgcagagtctagactcgtggtggacttctctcaattttctagggggaactaccgtgtgtcttggccaaaattcgcagtccccaacctccaatcactcaccaacctcctgtcctccaacttgtcctggttatcgctggatgtttctgcggcgttttatcatcttcctcttcatcctgctgctatgcctcatcttcttgttggttcttctggattatcaaggtatgttgcccgtttgtcctctaattccaggatcatcaaccaccagcacgggaccctgcagaacctgcacgactcctgctcaaggaacctctatgtatccctcctgttgctgtacaaaaccttcggatggaaactgcacctgtattcccatcccatcatcctgggctttcggaaaattcctatgggagtgggcctcagcccgtttctcttggctcagtttactagtgccatttgttcagtggttcgtagggctttcccccactgtttggctttcagttatatggatgatgtggtattgggggccaagtctgtacagcaccttgagtccctttttaccgctgttaccaattttcttttgtctttgggtatacatttaaaccctaacaaaacaaaaagatggggttattctctaaatttcatgggctatgtcattggaagttgg

SEQ ID NO: 118 - DNA, 900 bp, Hepatitis B virus
  ref <308>: AB205191
  ref <309>: 2006-01-12
  ref <313>: (1)..(900)
ttccacaacattccaccaagctctgcaggatcccagagtaagaggcctgtattttcctgctggtggctccagttccggaacagtgaaccctgttccgactactgcctcactcatctcgtcaatcttctcgaggattggggaccctgcaccgaacatggaaggcatcacatcaggattcctaggacccctgctcgtgttacaggcggggtttttcttgttgacaaaaatcctcacaataccgcagagtctagactcgtggtggacttctctcaattttctagggggagctcccgtgtgtcttggccaaaattcgcagtccccaacctccaatcactcaccaacctcttgtcctccaatttgtcctggctatcgctggatgtgtctgcggcgttttatcatcttcctcttcatcctgctgctatgcctcatcttcttgttggttcttctggactatcaaggtatgttgcccgtttgtcctctaattccaggatcatcaaccaccagtacgggaccctgccgaacctgcacgactcttgctcaaggaacctctatgtttccctcatgttgctgttcaaaaccttcggacggaaattgcacttgtattcccatcccatcatcatgggctttcggaaaattcctatgggagtgggcctcagcccgtttctcctggctcagtttactagtgccatttgttcagtggttcgccgggctttcccccactgtctggctttcagttatatggatgatgtggtattgggggccaagtctgtacaacatcttgagtccctttataccgctgttaccaattttcttttgtctttgggtatacatttaaatccaaacaaaacaaaaagatggggatattccctaaatttcatgggttatgtaattggaagttgg

SEQ ID NO: 119 - DNA, 900 bp, Hepatitis B virus
  ref <308>: AY090459
  ref <309>: 2002-08-07
  ref <313>: (1)..(900)
gaactcaactcagttccaccaggctctgttagatccgagggtaagggctctgtattttcctgctggtggctccagttcagagacacagaaccctgctccgactattgcctctctcacatcatcaatcttcttgaagactgggggccctgctatgaacatggacaacatcacatcaggactcctaggacccctgctcgtgttacaggcggtgtgtttcttgttgacaaaaatcctcacaataccacagagtctagactcgtggtggacttctctcaattttctagggggaacaccagggtgtcctggccaaaattcgcagtccccaacctccaatcacttaccaacctcctgtcctccaacttgtcctggttatcgctggatgtgtctgcggcgttttatcatcttcctcttcatcctgctgctatgcctcatcttcttgttggttcttctggactatcaaggtatgttgcccgtttgtcctctacttccaggatccacgaccaccagcacgggaccatgcaaaacctgcacaactcttgctcaaggaacctctatgtttccctcctgctgctgttccaaaccttcggacggaaactgcacttgtattcccatcccatcatcctgggctttaggaaaatacctatgggagtgggcctcagcccgtttctcctggctcagtttactagtgcaatttgttcagtggtgcgtagggctttcccccactgtttggcttttagttatatggatgatctggtattgggggccaaatctgtgcagcatcttgagtccctttataccgctgttaccaattttctgttatctgtgggtatccatttaaatacctctaaaacgaaaagatggggctatactttaaatttcatgggatatgttattggcagt

SEQ ID NO: 120 - DNA, 900 bp, Hepatitis B virus
  ref <308>: AF223963
  ref <309>: 2001-01-17
  ref <313>: (1)..(900)
ctccactcagttccaccaggctctgttagatccgagggtaagggctctgtattttcctgctggtggctccagttcagagacacagaaccctgctccgactattgcctctctcacatcatcaatcttcttgaagactgggggccctgctacgaacatggacaacatcacatcaggactcctaggacccctgctcgtgttacaggcggtgtgtttcttgttgacaaaaatcctcacaataccacagagtctagactcgtggtggacttctctcaattttctagggggaacacccgggtgtcctggccaaaattcgcagtccccaacctccaatcacttaccaacctcctgtcctccaacttgtcctggctatcgctggatgtgtctgcggcgttttatcatcttcctcttcatcctgctgctatgcctcatcttcttgttggttcttgtggactatcaaggtatgttgcccgtttgtcctccacttccaggatccacgaccaccagcacgggaccatgcaaaacctgcacaactcttgctcaaggaacctctatgtttccctcttgctgctgttccaaaccctcggacggaaactgcacttgtattcccatcccatcatcctgggctttaggaaaatacctatgggagtgggcctcagcccgtttctcctggctcagtttactagtgcaatttgttcagtggtgcgtagggctttcccccactgtctggcttttagttatatggatgatctggtattgggggccaaatctgtgcagcatcttgagtccctttataccgctgttaccaattttctgttatctgtgggtatccatttaaatacctcgaaaacaaaaagatggggttataccctaaatttcatgggttatgttattggcagttgg

SEQ ID NO: 121 - DNA, 900 bp, Hepatitis B virus
  ref <308>: AY311369
  ref <309>: 2006-08-28
  ref <313>: (1)..(900)
ctcaacccagttccaccaggctctgttggatcccagggtaagggctctgtacttccctgctggtggctccagttcagggacacagaaccctgctccgactattgcctctctcacatcatcaatcttctcgaagactgggggccctgctatgaacatggacaacattacatcaggactcctaggacccctgctcgtgttacaggcggtgtgtttcttgttgacaaaaatcctcacaataccacagagtctagactcgtggtggacttctctcaattttctagggggactacccgggtgtcctggccaaaattcgcagtccccaacctccaatcacttaccaacctcctgtcctccaacttgtcctggctatcgttggatgtgtctgcggcgttttatcatcttcctcttcatcctgctgctatgcctcatcttcttgttggttcttctggactatcaaggtatgttgcccgtttgtcctctacttccaggatccacgaccaccagcacgggaccctgcaaaacctgcacaactcttgcacaaggaacctctatgtttccctcctgttgctgttccaaaccctcggacggaaactgcacttgtattcccatcccatcatcttgggctttaggaaaatacctatgggagtgggcctcagcccgtttctcctggctcagtttactagtgcaatttgttcagtggtgcgtcgggctttcccccactgtttggcttttagttatatggatgatctggtattgggggccaaatctgtgcagcatcttgagtccctttataccgctgttaccaattttctgttatctgtgggtatccatttaaatacctctaaaacaaaaagatgggggtactccctacattttatgggctatgtcattggtagttgg

SEQ ID NO: 122 - DNA, 900 bp, Hepatitis B virus
  ref <308>: AB036915
  ref <309>: 2001-02-20
  ref <313>: (1)..(900)
ctcaacccagttccaccaggctctgttagatccgagggtaagggctctgtattttcctgctggtggctccagttcagggacacagaaccctgttccgactattgcctctctcacatcatcaatcttctcgaagactgggggccctgctatgaacatggagaacatcacatcaggactcctaggacccctgctcgtgttacaggcggtgtgtttcttgttgacaaaaatcctcacaataccacagagtctagactcgtggtggacttctctcaattttctagggggactacccgggtgtcctggccaaaattcgcagtccccaacctccaatcacttaccaacctcctgtcctccaacttgtcctggctatcgttggatgtgtctgcggcgttttatcatcttcctcttcatcctgctgctatgcctcatcttcttgttggttcttctggactatcaaggtatgttgcccgtttgtcctctacttccaggatccacaaccaccagcacgggaccatgcaaaacctgcacaactcttgctcaaggaacctctatgtttccctcctgttgctgttccaaaccctcggacggaaactgcacctgtattcccatcccatcatcttgggctttaggaaaatacctatgggagtgggcctcagcccgtttctcctggctcagtttactagtgcaatttgttcagtggtgcgtagggctttcccccactgtctggcttttagttatatggatgatctggtattgggggccaaatctgtgcagcatcttgagtccctttataccgctgttaccaattttttgttatctgtgggtatccatttaaatacttctaaaacaaaaagatggggttacaacctacatttcatgggttatgttattggtagttgg

SEQ ID NO: 123 - DNA, 900 bp, Hepatitis B virus
  ref <308>: AB166850
  ref <309>: 2010-02-09
  ref <313>: (1)..(900)
ctcaacccagttccaccaggccctgttggatccgagggtaagggctctgtctcctcctgctggtggctccagttcagagacacagaaccctgctccgactattgcctctctcacatcatcaatcttctcgaaaactgggggccctgctatgaacatggacaacatcacatcaggactcctaggacccctgctcgtgttacaggcggtgtgtttcttgttgacaaaaatccgcacaataccacagagtctagacttgtggtggacttctctcaattttctagggggactacccgggtgtcctggccaaaattcgcagtccccaacctccaatcacttaccaacctcctgtcctccaacttgtcctggctatcgttggatgtgtctgcggcgttttatcatcttcctcttcatcctgctgctatgcctcatcttcttgttggttcttctggactatcaaggtatgttgcccgtttgtcctctaattccaggatctacgaccaccagcacgggaccatgcaaaacctgcacaactcttgctcaaggaacctctatgtttccctcctgttgctgttcaaaaccttcggacggaaactgcacctgtattcccatcccatcatcttgggctttaggaaaatacctatgggagtgggcctcagcccgtttctcctggctcagtttactagtgcaatttgttcagtggtgcgtagggctttcccccactgtctggcttttagttatatggatgatctggtattgggggccaaatctgtgcagcatcttgagtccctttataccgctgttaccaattttctgttatctgtgggtatccatttgaatacctctaaaacaaaaagatggggttacaatttacatttcatgggttatatcattggtagttgg

SEQ ID NO: 124 - DNA, 900 bp, Hepatitis B virus
  ref <308>: AB064312
  ref <309>: 2002-06-04
  ref <313>: (1)..(900)
ctctacagcattccaccaagctctacaaaatcccacagtcaggggcctgtatcttcctgctggtggctccagttcagggatagtgaaccctgttccgactattgcctctcacatctcgtcaatcttctccaggattggggaccctgcaccgaacatggagaacatcacatcaggattcctaggacccctgctcgtgttacaggcggggtttttcttgttgacaagaatcctcacaataccgcagagtctagactcgtggtggacttctctcaattttctagggggagtgcccgtgtgtcctggcctaaattcgcagtccccaacctccaatcactcaccaatctcctgtcctccaacttgtcctggctatcgctggatgtgtctgcggcgttttatcatattcctcttcatcctgctgctatgcctcatcttcttgttggttcttctggactatcaaggtatgttgcccgtttgtcctctgattccaggatcctcgaccaccagtacgggaccctgcaaaacctgcacgactcctgctcaaggcaactctatgtatccctcatgttgctgtacaaaaccttcggacggaaattgcacctgtattcccatcccatcatcttgggctttcgcaaaatacctatgggagtgggcctcagtccgtttctcttggctcagtttactagtgccatttgttcagtggttcgtagggctttcccccactgtctggctttcagctatatggatgatgtggtattgggggccaaatctgtacaacatcttgagtccctttataccgctgttaccaattttcttttgtctttgggtatacatctaaaccctgacaaaacaaaaagatggggttattccttaaattttatgggatatgtaattggaagttgg

SEQ ID NO: 125 - DNA, 900 bp, Hepatitis B virus
  ref <308>: AB059659
  ref <309>: 2002-12-04
  ref <313>: (1)..(900)
ctcaacacagttccaccaagcactgttagatccgagagtaaggggtctgtattttcctgctggtggctccagttcagaaacacagaaccctgctccgactattgcctctctcacatcatcaatcttctcgaagactggggaccctgctatgaacatggagaacatcacatcaggactcctaggaccccttcccgtgttacagggggtgtttttctcgttgacaaaaatcctcacaataccacagagtctagactcgtggtggacttctctcaattttctagaggtaccacccgggtgtcctggccaaaattcgcagtccccaatctccaatcacttaccaacctcctgtcctccaacttgtcctggctatcgttggatgtgtctgcggcgttttatcatcttcctcttcatcctgctgctatgcctcatcttcttgttggttcttctggactatcaaggtatgttgcccgtgtgtcctctacttccaggatctacaaccaccagcacgggaccctgcaaaacctgcaccactcttgctcaaggaacctctatgtttccctcctgctgctgtaccaaaccttcggacggaaattgcacctgtattcccatcccatcatcttgggctttcggaaaatacctatgggagtgggcctcagcccgtttctcttggctcagtttactagtgcaatttgttcagtggtgcgtagggctttcccccactgtctggcttttagttatatggatgatttggtattgggggccaaatctgtgcagcatcttgagtccctttataccgctgttaccaattttttgttatctgtgggcatccatttgaacacagctaaaacaaaaaggtggggttattccttacactttatgggttatataattgggagttgg